European Patent Application EP 4 744 681 A1, published May 20, 2026. Title: 靶向靶细胞的复合物及其应用. Applicant: 上海宝济药业股份有限公司. Application CN. The sequence listing filed with the application follows.

SEQUENCE LISTING (71 sequences)

SEQ ID NO: 1 - protein, 214 aa, synthetic construct
DIQMTQSPSSLSASVGDRVTITCRASQDVSTAVAWYQQKPGKAPKLLIYSASYLYSGVPSRFSGSRSGTDFTLTISSLQPEDFATYYCQQHYTTPPTFGQGTKVEIKRTVAAPSVFIFPPSDEQLKSGTASVVCLLNNFYPREAKVQWKVDNALQSGNSQESVTEQDSKDSTYSLSSTLTLSKADYEKHKVYACEVTHQGLSSPVTKSFNRGEC

SEQ ID NO: 2 - protein, 450 aa, synthetic construct
EVQLVESGGGLVQPGGSLRLSCAASGFNIKDTYIHWVRQAPGKGLEWVARIYPTNGYTRYADSVKGRFTISADTSKNTAYLQMNSLRAEDTAVYYCSRWGGEGFYAMDYWGQGTLVTVSSASTKGPSVFPLAPSSKSTSGGTAALGCLVKDYFPEPVTVSWNSGALTSGVHTFPAVLQSSGLYSLSSVVTVPSSSLGTQTYICNVNHKPSNTKVDKKVEPKSCDKTHTCPPCPAPELLGGPSVFLFPPKPKDTLMISRTPEVTCVVVDVSHEDPEVKFNWYVDGVEVHNAKTKPREEQYNSTYRVVSVLTVLHQDWLNGKEYKCKVSNKALPAPIEKTISKAKGQPREPQVYTLPPCREEMTKNQVSLWCLVKGFYPSDIAVEWESNGQPENNYKTTPPVLDSDGSFFLYSKLTVDKSRWQQGNVFSCSVMHEALHNHYTQKSLSLSPGK

SEQ ID NO: 3 - protein, 449 aa, synthetic construct
EVQLVESGGGLVQPGGSLRLSCAASGFTFTDYTMDWVRQAPGKGLEWVADVNPNSGGSILNRRFKGRFTLSVDRSKNTLYLQMNSLRAEDTAVYYCARNLGPLFYFDYWGQGTLVTVSSASTKGPSVFPLAPSSKSTSGGTAALGCLVKDYFPEPVTVSWNSGALTSGVHTFPAVLQSSGLYSLSSVVTVPSSSLGTQTYICNVNHKPSNTKVDKKVEPKSCDKTHTCPPCPAPELLGGPSVFLFPPKPKDTLMISRTPEVTCVVVDVSHEDPEVKFNWYVDGVEVHNAKTKPREEQYNSTYRVVSVLTVLHQDWLNGKEYKCKVSNKALPAPIEKTISKAKGQPREPQVCTLPPSREEMTKNQVSLSCAVKGFYPSDIAVEWESNGQPENNYKTTPPVLDSDGSFFLVSKLTVDKSRWQQGNVFSCSVMHEALHNHYTQKSLSLSPGK

SEQ ID NO: 4 - protein, 380 aa, synthetic construct
DASLPYLQKESVFQSGAHAYRIPALLYLPGQQSLLAFAEQRRSKKDEHAELIVLRRGDYDAGTHQVQWQAQEVVAQARLDGHRSMNPCPLYDEQTGTLFLFFIAIPGQVTEQQQLQTRANVTRLCYVTSTDHGRTWSSPRDLTDAAIGPAYREWSTFAVGPGHCLQLHDRARSLVVPAYAYRKLHPKQRPIPSAFCFLSHDHGRTWARGHFVAQDTLECQVAEVETGEQRVVTLNARSHLRFRVQAQSTNDGLDFQESQLVKKLVEPPPTGCQGSVISFPSPRSGPGSPAQWLLYTHPTHSWQRADLGAYLNPRPPAPEAWSEPVLLAKGSAAYSDLQSMGTGPDGSPLFGCLYEANDYEEIVFLMFTLKQAFPAEYLPQ

SEQ ID NO: 5 - protein, 380 aa, synthetic construct
MASLPVLQKESVFQSGAHAYRIPALLYLPGQQTLLAFAEQRASKKDEHAELIVLRRGDYDAPTHQVQWQAQEVVAQARLDGHRSMNPCPLYDAQTETLFLFFIAIPGQVTEQQQLQTRANVTRLCQVTSTDHGRTWSSPRDLTDAAIGPAYQEWSTFAVGPGHCLQLHDRARSLVVPAYAYRKLHPIQRPSPSAFCFLSHDHGHTWVRGHFVAQDTLECQVAEVETGEQRVVTLNARSHLQARVQAQSTNDGFDFQESQLVKKLVEPPPQGCQGSVISFPSPRSGPGSPAQWLLYTHPTHSWQRADLGAYLNPRPPAPEAWSEPVLLAKGSCAYSDLQSMGTGPDGSPLFGCLYEANDYEEIVFLMFTLKQAFPAEYLPQ

SEQ ID NO: 6 - protein, 447 aa, synthetic construct [sequence omitted]

SEQ ID NO: 7 - protein, 414 aa, synthetic construct
FRGPLLPNRPFTTVWNANTQWCLERHGVDVDVSVFDVVANPGQTFRGPDMTIFYSSQLGTYPYYTPTGEPVFGGLPQNASLIAHLARTFQDILAAIPAPDFSGLAVIDWEAWRPRWAFNWDTKDIYRQRSRALVQAQHPDWPAPQVEAVAQDQFQGAARAWMAGTLQLGRALRPRGLWGFYGFPDCYNYDFLSPNYTGQCPSGIRAQNDQLGWLWGQSRALYPSIYMPAVLEGTGKSQMYVQHRVAEAFRVAVAAGDPNLPVLPYVQIFYDTTNHFLPLDELEHSLGESAAQGAAGVVLWVSWENTRTKESCQAIKEYMDTTLGPFILNVTSGALLCSQALCSGHGRCVRRTSHPKALLLLNPASFSIQLTPGGGPLSLRGALSLEDQAQMAVEFKCRCYPGWQAPWCERKSMW

SEQ ID NO: 8 - protein, 1021 aa, synthetic construct
MKRKCLSKRLMLAITMATIFTVNSTLPIYAAVDKNNATAAVQNESKRYTVSYLKTLNYYDLVDLLVKTEIENLPDLFQYSSDAKEFYGNKTRMSFIMDEIGRRAPQYTEIDHKGIPTLVEVVRAGFYLGFHNKELNEINKRSFKERVIPSILAIQKNPNFKLGTEVQDKIVSATGLLAGNETAPPEVVNNFTPILQDCIKNIDRYALDDLKSKALFNVLAAPTYDITEYLRATKEKPENTPWYGKIDGFINELKKLALYGKINDNNSWIIDNGIYHIAPLGKLHSNNKIGIETLTEVMKVYPYLSMQHLQSADQIKRHYDSKDAEGNKIPLDKFKKEGKEKYCPKTYTFDDGKVIIKAGARVEEEKVKRLYWASKEVNSQFFRVYGIDKPLEEGNPDDILTMVIYNSPEEYKLNSVLYGYDTNNGGMYIEPEGTFFTYEREAQESTYTLEELFRHEYTHYLQGRYAVPGQWGRTKLYDNDRLTWYEEGGAELFAGSTRTSGILPRKSIVSNIHNTTRNNRYKLSDTVHSKYGASFEFYNYACMFMDYMYNKDMGILNKLNDLAKNNDVDGYDNYIRDLSSNYALNDKYQDHMQERIDNYENLTVPFVADDYLVRHAYKNPNEIYSEISEVAKLKDAKSEVKKSQYFSTFTLRGSYTGGASKGKLEDQKAMNKFIDDSLKKLDTYSWSGYKTLTAYFTNYKVDSSNRVTYDVVFHGYLPNEGDSKNSLPYGKINGTYKGTEKEKIKFSSEGSFDPDGKIVSYEWDFGDGNKSNEENPEHSYDKVGTYTVKLKVTDDKGESSVSTTTAEIKDLSENKLPVIYMHVPKSGALNQKVVFYGKGTYDPDGSIAGYQWDFGDGSDFSSEQNPSHVYTKKGEYTVTLRVMDSSGQMSEKTMKIKITDPVYPIGTEKEPNNSKETASGPIVPGIPVSGTIENTSDQDYFYFDVITPGEVKIDINKLGYGGATWVVYDENNNAVSYATDDGQNLSGKFKADKPGRYYIHLYMFNGSYMPYRINIEGSVGR

SEQ ID NO: 9 - protein, 644 aa, synthetic construct
MQSSSITRKDFDHINLEYSGLEKVNKAVAAGNYDDAAKALLAYYREKSKAREPDFSNAEKPADIRQPIDKVTREMADKALVHQFQPHKGYGYFDYGKDINWQMWPVKDNEVRWQLHRVKWWQAMALVYHATGDEKYAREWVYQYSDWARKNPLGLSQDNDKFVWRPLEVSDRVQSLPPTFSLFVNSPAFTPAFLMEFLNSYHQQADYLSTHYAEQGNHRLFEAQRNLFAGVSFPEFKDSPRWRQTGISVLNTEIKKQVYADGMQFELSPIYHVAAIDIFLKAYGSAKRVNLEKEFPQSYVQTVENMIMALISISLPDYNTPMFGDSWITDKNFRMAQFASWARVFPANQAIKYFATDGKQGKAPNFLSKALSNAGFYTFRSGWDKNATVMVLKASPPGEFHAQPDNGTFELFIKGRNFTPDAGVFVYSGDEAIMKLRNWYRQTRIHSTLTLDNQNMVITKARQNKWETGNNLDVLTYTNPSYPNLDHQRSVLFINKKYFLVIDRAIGEATGNLGVHWQLKEDSNPVFDKTKNRVYTTYRDGNNLMIQSLNADRTSLNEEEGKVSYVYNKELKRPAFVFEKPKKNAGTQNFVSIVYPYDGQKAPEISIRENKGNDFEKGKLNLTLTINGKQQLVLVPWSHPQFEK

SEQ ID NO: 10 - protein, 678 aa, synthetic construct
QQTGTAELIMKRVMLDLKKPLRNMDKVAEKDLNTLQPDGSWKDVPYKDDAMTNWLPNNHLLQLETIIQAYIEKDSHYYGDDKVFDQISKAFKYWYDSDPKSRNWWHNEIATPQALGEMLILMRYGKKPLDEALVHKLTERMKRGEPEKKTGANKTDIALHYFYRALLTSDEALLSFAVKELFYPVQFVHYEEGLQYDYSYLQHGPQLQISSYGAVFITGVLKLANYVRDTPYALSTEKLAIFSKYYRDSYLKAIRGSYMDFNVEGRGVSRPDILNKKAEKKRLLVAKMIDLKHTEEWADAIARTDSTVAAGYKIEPYHHQFWNGDYVQHLRPAYSFNVRMVSKRTRRSESGNKENLLGRYLSDGATNIQLRGPEYYNIMPVWEWDKIPGITSRDYLTDRPLTKLWGEQGSNDFAGGVSDGVYGASAYALDYDSLQAKKAWFFFDKEIVCLGAGINSNAPENITTTLNQSWLNGPVISTAGKTGRGKITTFKAQGQFWLLHDAIGYYFPEGANLSLSTQSQKGNWFHINNSHSKDEVSGDVFKLWINHGARPENAQYAYIVLPGINKPEEIKKYNGTAPKVLANTNQLQAVYHQQLDMVQAIFYTAGKLSVAGIEIETDKPCAVLIKHINGKQVIWAADPLQKEKTAVLSIRDLKTGKTNRVKIDFPQQEFAGATVELK

SEQ ID NO: 11 - protein, 1021 aa, synthetic construct
MPIFRFTALAMTLGLLSAPYNAMAATSNPAFDPKNLMQSEIYHFAQNNPLADFSSDKNSILTLSDKRSIMGNQSLLWKWKGGSSFTLHKKLIVPTDKEASKAWGRSSTPVFSFWLYNEKPIDGYLTIDFGEKLISTSEAQAGFKVKLDFTGWRAVGVSLNNDLENREMTLNATNTSSDGTQDSIGRSLGAKVDSIRFKAPSNVSQGEIYIDRIMFSVDDARYQWSDYQVKTRLSEPEIQFHNVKPQLPVTPENLAAIDLIRQRLINEFVGGEKETNLALEENISKLKSDFDALNIHTLANGGTQGRHLITDKQIIIYQPENLNSQDKQLFDNYVILGNYTTLMFNISRAYVLEKDPTQKAQLKQMYLLMTKHLLDQGFVKGSALVTTHHWGYSSRWWYISTLLMSDALKEANLQTQVYDSLLWYSREFKSSFDMKVSADSSDLDYFNTLSRQHLALLLLEPDDQKRINLVNTFSHYITGALTQVPPGGKDGLRPDGTAWRHEGNYPGYSFPAFKNASQLIYLLRDTPFSVGESGWNNLKKAMVSAWIYSNPEVGLPLAGRHPFNSPSLKSVAQGYYWLAMSAKSSPDKTLASIYLAISDKTQNESTAIFGETITPASLPQGFYAFNGGAFGIHRWQDKMVTLKAYNTNVWSSEIYNKDNRYGRYQSHGVAQIVSNGSQLSQGYQQEGWDWNRMQGATTIHLPLKDLDSPKPHTLMQRGERGFSGTSSLEGQYGMMAFDLIYPANLERFDPNFTAKKSVLAADNHLIFIGSNINSSDKNKNVETTLFQHAITPTLNTLWINGQKIENMPYQTTLQQGDWLIDSNGNGYLITQAEKVNVSRQHQVSAENKNRQPTEGNFSSAWIDHSTRPKDASYEYMVFLDATPEKMGEMAQKFRENNGLYQVLRKDKDVHIILDKLSNVTGYAFYQPASIEDKWIKKVNKPAIVMTHRQKDTLIVSAVTPDLNMTRQKAATPVTINVTINGKWQSADKNSEVKYQVSGDNTELTFTSYFGIPQEIKLSPLP

SEQ ID NO: 12 - protein, 126 aa, synthetic construct
QVQLVESGGGLVQAGGSLNLSCAVSDIMFSWSTMGWYRQAPGKERELVAQERGSGRINYADFVKGRFTISRDSAKNTMNLQMNSLKPEDTGVYYCWVRRPSGSWRGQHYPDAQEYWGQGTQVTVSS

SEQ ID NO: 13 - protein, 365 aa, synthetic construct
MGVPRPQPWALGLLLFLLPGSLGAESHLSLLYHLTAVSSPAPGTPAFWVSGWLGPQQYLSYNSLRGEAEPCGAWVWENQVSWYWEKETTDLRIKEKLFLEAFKALGGKGPYTLQGLLGCELGPDNTSVPTAKFALNGEEFMNFDLKQGTWGGDWPEALAISQRWQQQDKAANKELTFLLFSCPHRLREHLERGRGNLEWKEPPSMRLKARPSSPGFSVLTCSAFSFYPPELQLRFLRNGLAAGTGQGDFGPNSDGSFHASSSLTVKSGDEHHYCCIVQHAGLAQPLRVELESPAKSSVLVVGIVIGVLLLTAAAVGGALLWRRMRSGLPAPWISLRGDDTGVLLPTPGEAQDADLKDVNVIPATA

SEQ ID NO: 14 - protein, 508 aa, synthetic construct
MKKKNIYSIRKLGVGIASVTLGTLLISGGVTPAANAAQHDEAQQNAFYQVLNMPNLNADQRNGFIQSLKDDPSQSANVLGEAQKLNDSQAPKADAQQNKFNKDQQSAFYEILNMPNLNEEQRNGFIQSLKDDPSQSTNVLGEAKKLNESQAPKADNNFNKEQQNAFYEILNMPNLNEEQRNGFIQSLKDDPSQSANLLAEAKKLNESQAPKADNKFNKEQQNAFYEILHLPNLNEEQRNGFIQSLKDDPSQSANLLAEAKKLNDAQAPKADNKFNKEQQNAFYEILHLPNLTEEQRNGFIQSLKDDPSVSKEILAEAKKLNDAQAPKEEDNNKPGKEDGNKPGKEDGNKPGKEDNKKPGKEDGNKPGKEDNKKPGKEDGNKPGKEDGNKPGKEDGNKPGKEDGNKPGKEDGNGVHVVKPGDTVNDIAKANGTTADKIAADNKLADKNMIKPGQELVVDKKQPANHADANKAQALPETGEENPFIGTTVFGGLSLALGAALLAGRRREL

SEQ ID NO: 15 - protein, 593 aa, synthetic construct
MEKEKKVKYFLRKSAFGLASVSAAFLVGSTVFAVDSPIEDTPIIRNGGELTNLLGNSETTLALRNEESATADLTAAAVADTVAAAAAENAGAAAWEAAAAADALAKAKADALKEFNKYGVSDYYKNLINNAKTVEGVKDLQAQVVESAKKARISEATDGLSDFLKSQTPAEDTVKSIELAEAKVLANRELDKYGVSDYHKNLINNAKTVEGVKDLQAQVVESAKKARISEATDGLSDFLKSQTPAEDTVKSIELAEAKVLANRELDKYGVSDYYKNLINNAKTVEGVKALIDEILAALPKTDTYKLILNGKTLKGETTTEAVDAATAEKVFKQYANDNGVDGEWTYDDATKTFTVTEKPEVIDASELTPAVTTYKLVINGKTLKGETTTEAVDAATAEKVFKQYANDNGVDGEWTYDDATKTFTVTEKPEVIDASELTPAVTTYKLVINGKTLKGETTTKAVDAETAEKAFKQYANDNGVDGVWTYDDATKTFTVTEMVTEVPGDAPTEPEKPEASIPLVPLTPATPIAKDDAKKDDTKKEDAKKPEAKKEDAKKAETLPTTGEGSNPFFTAAALAVMAGAGALAVASKRKED

SEQ ID NO: 16 - protein, 12 aa, synthetic construct
EPIHRSTLTALL

SEQ ID NO: 17 - protein, 10 aa, synthetic construct
TWKTSRISIF

SEQ ID NO: 18 - protein, 33 aa, synthetic construct
FNMQQQRRFYEALHDPNLNEEQRNAKIKSIRDD

SEQ ID NO: 19 - protein, 565 aa, synthetic construct
FRGPLLPNRPFTTVWNANTQWCLERHGVDVDVSVFDVVANPGQTFRGPDMTIFYSSQLGTYPYYTPTGEPVFGGLPQNASLIAHLARTFQDILAAIPAPDFSGLAVIDWEAWRPRWAFNWDTKDIYRQRSRALVQAQHPDWPAPQVEAVAQDQFQGAARAWMAGTLQLGRALRPRGLWGFYGFPDCYNYDFLSPNYTGQCPSGIRAQNDQLGWLWGQSRALYPSIYMPAVLEGTGKSQMYVQHRVAEAFRVAVAAGDPNLPVLPYVQIFYDTTNHFLPLDELEHSLGESAAQGAAGVVLWVSWENTRTKESCQAIKEYMDTTLGPFILNVTSGALLCSQALCSGHGRCVRRTSHPKALLLLNPASFSIQLTPGGGPLSLRGALSLEDQAQMAVEFKCRCYPGWQAPWCERKSMWGGGGSGGGGSGGGGSGGGGSGGGGSQVQLVESGGGLVQAGGSLNLSCAVSDIMFSWSTMGWYRQAPGKERELVAQERGSGRINYADFVKGRFTISRDSAKNTMNLQMNSLKPEDTGVYYCWVRRPSGSWRGQHYPDAQEYWGQGTQVTVSS

SEQ ID NO: 20 - protein, 598 aa, synthetic construct
LNFRAPPVIPNVPFLWAWNAPSEFCLGKFDEPLDMSLFSFIGSPRINATGQGVTIFYVDRLGYYPYIDSITGVTVNGGIPQKISLQDHLDKAKKDITFYMPVDNLGMAVIDWEEWRPTWARNWKPKDVYKNRSIELVQQQNVQLSLTEATEKAKQEFEKAGKDFLVETIKLGKLLRPNHLWGYYLFPDCYNHHYKKPGYNGSCFNVEIKRNDDLSWLWNESTALYPSIYLNTQQSPVAATLYVRNRVREAIRVSKIPDAKSPLPVFAYTRIVFTDQVLKFLSQDELVYTFGETVALGASGIVIWGTLSIMRSMKSCLLLDNYMETILNPYIINVTLAAKMCSQVLCQEQGVCIRKNWNSSDYLHLNPDNFAIQLEKGGKFTVRGKPTLEDLEQFSEKFYCSCYSTLSCKEKADVKDTDAVDVCIADGVCIDAFLKPPMETEEPQIFYGGGGSGGGGSGGGGSGGGGSGGGGSQVQLVESGGGLVQAGGSLNLSCAVSDIMFSWSTMGWYRQAPGKERELVAQERGSGRINYADFVKGRFTISRDSAKNTMNLQMNSLKPEDTGVYYCWVRRPSGSWRGQHYPDAQEYWGQGTQVTVSS

SEQ ID NO: 21 - protein, 565 aa, synthetic construct
QVQLVESGGGLVQAGGSLNLSCAVSDIMFSWSTMGWYRQAPGKERELVAQERGSGRINYADFVKGRFTISRDSAKNTMNLQMNSLKPEDTGVYYCWVRRPSGSWRGQHYPDAQEYWGQGTQVTVSSGGGGSGGGGSGGGGSGGGGSGGGGSFRGPLLPNRPFTTVWNANTQWCLERHGVDVDVSVFDVVANPGQTFRGPDMTIFYSSQLGTYPYYTPTGEPVFGGLPQNASLIAHLARTFQDILAAIPAPDFSGLAVIDWEAWRPRWAFNWDTKDIYRQRSRALVQAQHPDWPAPQVEAVAQDQFQGAARAWMAGTLQLGRALRPRGLWGFYGFPDCYNYDFLSPNYTGQCPSGIRAQNDQLGWLWGQSRALYPSIYMPAVLEGTGKSQMYVQHRVAEAFRVAVAAGDPNLPVLPYVQIFYDTTNHFLPLDELEHSLGESAAQGAAGVVLWVSWENTRTKESCQAIKEYMDTTLGPFILNVTSGALLCSQALCSGHGRCVRRTSHPKALLLLNPASFSIQLTPGGGPLSLRGALSLEDQAQMAVEFKCRCYPGWQAPWCERKSMW

SEQ ID NO: 22 - protein, 598 aa, synthetic construct
QVQLVESGGGLVQAGGSLNLSCAVSDIMFSWSTMGWYRQAPGKERELVAQERGSGRINYADFVKGRFTISRDSAKNTMNLQMNSLKPEDTGVYYCWVRRPSGSWRGQHYPDAQEYWGQGTQVTVSSGGGGSGGGGSGGGGSGGGGSGGGGSLNFRAPPVIPNVPFLWAWNAPSEFCLGKFDEPLDMSLFSFIGSPRINATGQGVTIFYVDRLGYYPYIDSITGVTVNGGIPQKISLQDHLDKAKKDITFYMPVDNLGMAVIDWEEWRPTWARNWKPKDVYKNRSIELVQQQNVQLSLTEATEKAKQEFEKAGKDFLVETIKLGKLLRPNHLWGYYLFPDCYNHHYKKPGYNGSCFNVEIKRNDDLSWLWNESTALYPSIYLNTQQSPVAATLYVRNRVREAIRVSKIPDAKSPLPVFAYTRIVFTDQVLKFLSQDELVYTFGETVALGASGIVIWGTLSIMRSMKSCLLLDNYMETILNPYIINVTLAAKMCSQVLCQEQGVCIRKNWNSSDYLHLNPDNFAIQLEKGGKFTVRGKPTLEDLEQFSEKFYCSCYSTLSCKEKADVKDTDAVDVCIADGVCIDAFLKPPMETEEPQIFY

SEQ ID NO: 23 - protein, 1606 aa, synthetic construct
MKRKCLSKRLMLAITMATIFTVNSTLPIYAAVDKNNATAAVQNESKRYTVSYLKTLNYYDLVDLLVKTEIENLPDLFQYSSDAKEFYGNKTRMSFIMDEIGRRAPQYTEIDHKGIPTLVEVVRAGFYLGFHNKELNEINKRSFKERVIPSILAIQKNPNFKLGTEVQDKIVSATGLLAGNETAPPEVVNNFTPILQDCIKNIDRYALDDLKSKALFNVLAAPTYDITEYLRATKEKPENTPWYGKIDGFINELKKLALYGKINDNNSWIIDNGIYHIAPLGKLHSNNKIGIETLTEVMKVYPYLSMQHLQSADQIKRHYDSKDAEGNKIPLDKFKKEGKEKYCPKTYTFDDGKVIIKAGARVEEEKVKRLYWASKEVNSQFFRVYGIDKPLEEGNPDDILTMVIYNSPEEYKLNSVLYGYDTNNGGMYIEPEGTFFTYEREAQESTYTLEELFRHEYTHYLQGRYAVPGQWGRTKLYDNDRLTWYEEGGAELFAGSTRTSGILPRKSIVSNIHNTTRNNRYKLSDTVHSKYGASFEFYNYACMFMDYMYNKDMGILNKLNDLAKNNDVDGYDNYIRDLSSNYALNDKYQDHMQERIDNYENLTVPFVADDYLVRHAYKNPNEIYSEISEVAKLKDAKSEVKKSQYFSTFTLRGSYTGGASKGKLEDQKAMNKFIDDSLKKLDTYSWSGYKTLTAYFTNYKVDSSNRVTYDVVFHGYLPNEGDSKNSLPYGKINGTYKGTEKEKIKFSSEGSFDPDGKIVSYEWDFGDGNKSNEENPEHSYDKVGTYTVKLKVTDDKGESSVSTTTAEIKDLSENKLPVIYMHVPKSGALNQKVVFYGKGTYDPDGSIAGYQWDFGDGSDFSSEQNPSHVYTKKGEYTVTLRVMDSSGQMSEKTMKIKITDPVYPIGTEKEPNNSKETASGPIVPGIPVSGTIENTSDQDYFYFDVITPGEVKIDINKLGYGGATWVVYDENNNAVSYATDDGQNLSGKFKADKPGRYYIHLYMFNGSYMPYRINIEGSVGRGGGGSGGGGSGGGGSGGGGSGGGGSVDSPIEDTPIIRNGGELTNLLGNSETTLALRNEESATADLTAAAVADTVAAAAAENAGAAAWEAAAAADALAKAKADALKEFNKYGVSDYYKNLINNAKTVEGVKDLQAQVVESAKKARISEATDGLSDFLKSQTPAEDTVKSIELAEAKVLANRELDKYGVSDYHKNLINNAKTVEGVKDLQAQVVESAKKARISEATDGLSDFLKSQTPAEDTVKSIELAEAKVLANRELDKYGVSDYYKNLINNAKTVEGVKALIDEILAALPKTDTYKLILNGKTLKGETTTEAVDAATAEKVFKQYANDNGVDGEWTYDDATKTFTVTEKPEVIDASELTPAVTTYKLVINGKTLKGETTTEAVDAATAEKVFKQYANDNGVDGEWTYDDATKTFTVTEKPEVIDASELTPAVTTYKLVINGKTLKGETTTKAVDAETAEKAFKQYANDNGVDGVWTYDDATKTFTVTEMVTEVPGDAPTEPEKPEASIPLVPLTPATPIAKDDAKKDDTKKEDAKKPEAKKEDAKKAETLPTTGEGSNPFFTAAALAVMAGAGALAVASKRKED

SEQ ID NO: 24 - protein, 1033 aa, synthetic construct
QSSSITRKDFDHINLEYSGLEKVNKAVAAGNYDDAAKALLAYYREKSKAREPDFSNAEKPADIRQPIDKVTREMADKALVHQFQPHKGYGYFDYGKDINWQMWPVKDNEVRWQLHRVKWWQAMALVYHATGDEKYAREWVYQYSDWARKNPLGLSQDNDKFVWRPLEVSDRVQSLPPTFSLFVNSPAFTPAFLMEFLNSYHQQADYLSTHYAEQGNHRLFEAQRNLFAGVSFPEFKDSPRWRQTGISVLNTEIKKQVYADGMQFELSPIYHVAAIDIFLKAYGSAKRVNLEKEFPQSYVQTVENMIMALISISLPDYNTPMFGDSWITDKNFRMAQFASWARVFPANQAIKYFATDGKQGKAPNFLSKALSNAGFYTFRSGWDKNATVMVLKASPPGEFHAQPDNGTFELFIKGRNFTPDAGVFVYSGDEAIMKLRNWYRQTRIHSTLTLDNQNMVITKARQNKWETGNNLDVLTYTNPSYPNLDHQRSVLFINKKYFLVIDRAIGEATGNLGVHWQLKEDSNPVFDKTKNRVYTTYRDGNNLMIQSLNADRTSLNEEEGKVSYVYNKELKRPAFVFEKPKKNAGTQNFVSIVYPYDGQKAPEISIRENKGNDFEKGKLNLTLTINGKQQLVLVPWSHPQFEKGGGGSGGGGSGGGGSGGGGSGGGGSMGVPRPQPWALGLLLFLLPGSLGAESHLSLLYHLTAVSSPAPGTPAFWVSGWLGPQQYLSYNSLRGEAEPCGAWVWENQVSWYWEKETTDLRIKEKLFLEAFKALGGKGPYTLQGLLGCELGPDNTSVPTAKFALNGEEFMNFDLKQGTWGGDWPEALAISQRWQQQDKAANKELTFLLFSCPHRLREHLERGRGNLEWKEPPSMRLKARPSSPGFSVLTCSAFSFYPPELQLRFLRNGLAAGTGQGDFGPNSDGSFHASSSLTVKSGDEHHYCCIVQHAGLAQPLRVELESPAKSSVLVVGIVIGVLLLTAAAVGGALLWRRMRSGLPAPWISLRGDDTGVLLPTPGEAQDADLKDVNVIPATA

SEQ ID NO: 25 - protein, 1079 aa, synthetic construct
MPIFRFTALAMTLGLLSAPYNAMAATSNPAFDPKNLMQSEIYHFAQNNPLADFSSDKNSILTLSDKRSIMGNQSLLWKWKGGSSFTLHKKLIVPTDKEASKAWGRSSTPVFSFWLYNEKPIDGYLTIDFGEKLISTSEAQAGFKVKLDFTGWRAVGVSLNNDLENREMTLNATNTSSDGTQDSIGRSLGAKVDSIRFKAPSNVSQGEIYIDRIMFSVDDARYQWSDYQVKTRLSEPEIQFHNVKPQLPVTPENLAAIDLIRQRLINEFVGGEKETNLALEENISKLKSDFDALNIHTLANGGTQGRHLITDKQIIIYQPENLNSQDKQLFDNYVILGNYTTLMFNISRAYVLEKDPTQKAQLKQMYLLMTKHLLDQGFVKGSALVTTHHWGYSSRWWYISTLLMSDALKEANLQTQVYDSLLWYSREFKSSFDMKVSADSSDLDYFNTLSRQHLALLLLEPDDQKRINLVNTFSHYITGALTQVPPGGKDGLRPDGTAWRHEGNYPGYSFPAFKNASQLIYLLRDTPFSVGESGWNNLKKAMVSAWIYSNPEVGLPLAGRHPFNSPSLKSVAQGYYWLAMSAKSSPDKTLASIYLAISDKTQNESTAIFGETITPASLPQGFYAFNGGAFGIHRWQDKMVTLKAYNTNVWSSEIYNKDNRYGRYQSHGVAQIVSNGSQLSQGYQQEGWDWNRMQGATTIHLPLKDLDSPKPHTLMQRGERGFSGTSSLEGQYGMMAFDLIYPANLERFDPNFTAKKSVLAADNHLIFIGSNINSSDKNKNVETTLFQHAITPTLNTLWINGQKIENMPYQTTLQQGDWLIDSNGNGYLITQAEKVNVSRQHQVSAENKNRQPTEGNFSSAWIDHSTRPKDASYEYMVFLDATPEKMGEMAQKFRENNGLYQVLRKDKDVHIILDKLSNVTGYAFYQPASIEDKWIKKVNKPAIVMTHRQKDTLIVSAVTPDLNMTRQKAATPVTINVTINGKWQSADKNSEVKYQVSGDNTELTFTSYFGIPQEIKLSPLPGGGGSGGGGSGGGGSGGGGSGGGGSFNMQQQRRFYEALHDPNLNEEQRNAKIKSIRDD

SEQ ID NO: 26 - protein, 1258 aa, synthetic construct
QQTGTAELIMKRVMLDLKKPLRNMDKVAEKDLNTLQPDGSWKDVPYKDDAMTNWLPNNHLLQLETIIQAYIEKDSHYYGDDKVFDQISKAFKYWYDSDPKSRNWWHNEIATPQALGEMLILMRYGKKPLDEALVHKLTERMKRGEPEKKTGANKTDIALHYFYRALLTSDEALLSFAVKELFYPVQFVHYEEGLQYDYSYLQHGPQLQISSYGAVFITGVLKLANYVRDTPYALSTEKLAIFSKYYRDSYLKAIRGSYMDFNVEGRGVSRPDILNKKAEKKRLLVAKMIDLKHTEEWADAIARTDSTVAAGYKIEPYHHQFWNGDYVQHLRPAYSFNVRMVSKRTRRSESGNKENLLGRYLSDGATNIQLRGPEYYNIMPVWEWDKIPGITSRDYLTDRPLTKLWGEQGSNDFAGGVSDGVYGASAYALDYDSLQAKKAWFFFDKEIVCLGAGINSNAPENITTTLNQSWLNGPVISTAGKTGRGKITTFKAQGQFWLLHDAIGYYFPEGANLSLSTQSQKGNWFHINNSHSKDEVSGDVFKLWINHGARPENAQYAYIVLPGINKPEEIKKYNGTAPKVLANTNQLQAVYHQQLDMVQAIFYTAGKLSVAGIEIETDKPCAVLIKHINGKQVIWAADPLQKEKTAVLSIRDLKTGKTNRVKIDFPQQEFAGATVELKGGGGSGGGGSGGGGSGGGGSVDSPIEDTPIIRNGGELTNLLGNSETTLALRNEESATADLTAAAVADTVAAAAAENAGAAAWEAAAAADALAKAKADALKEFNKYGVSDYYKNLINNAKTVEGVKDLQAQVVESAKKARISEATDGLSDFLKSQTPAEDTVKSIELAEAKVLANRELDKYGVSDYHKNLINNAKTVEGVKDLQAQVVESAKKARISEATDGLSDFLKSQTPAEDTVKSIELAEAKVLANRELDKYGVSDYYKNLINNAKTVEGVKALIDEILAALPKTDTYKLILNGKTLKGETTTEAVDAATAEKVFKQYANDNGVDGEWTYDDATKTFTVTEKPEVIDASELTPAVTTYKLVINGKTLKGETTTEAVDAATAEKVFKQYANDNGVDGEWTYDDATKTFTVTEKPEVIDASELTPAVTTYKLVINGKTLKGETTTKAVDAETAEKAFKQYANDNGVDGVWTYDDATKTFTVTEMVTEVPGDAPTEPEKPEASIPLVPLTPATPIAKDDAKKDDTKKEDAKKPEAKKEDAKKAETLPTTGEGSNPFFTAAALAVMAGAGALAVASKRKED

SEQ ID NO: 27 - protein, 433 aa, synthetic construct
DASLPYLQKESVFQSGAHAYRIPALLYLPGQQSLLAFAEQRRSKKDEHAELIVLRRGDYDAGTHQVQWQAQEVVAQARLDGHRSMNPCPLYDEQTGTLFLFFIAIPGQVTEQQQLQTRANVTRLCYVTSTDHGRTWSSPRDLTDAAIGPAYREWSTFAVGPGHCLQLHDRARSLVVPAYAYRKLHPKQRPIPSAFCFLSHDHGRTWARGHFVAQDTLECQVAEVETGEQRVVTLNARSHLRFRVQAQSTNDGLDFQESQLVKKLVEPPPTGCQGSVISFPSPRSGPGSPAQWLLYTHPTHSWQRADLGAYLNPRPPAPEAWSEPVLLAKGSAAYSDLQSMGTGPDGSPLFGCLYEANDYEEIVFLMFTLKQAFPAEYLPQGGGGSGGGGSGGGGSGGGGSFNMQQQRRFYEALHDPNLNEEQRNAKIKSIRDD

SEQ ID NO: 28 - protein, 433 aa, synthetic construct
FNMQQQRRFYEALHDPNLNEEQRNAKIKSIRDDGGGGSGGGGSGGGGSGGGGSDASLPYLQKESVFQSGAHAYRIPALLYLPGQQSLLAFAEQRRSKKDEHAELIVLRRGDYDAGTHQVQWQAQEVVAQARLDGHRSMNPCPLYDEQTGTLFLFFIAIPGQVTEQQQLQTRANVTRLCYVTSTDHGRTWSSPRDLTDAAIGPAYREWSTFAVGPGHCLQLHDRARSLVVPAYAYRKLHPKQRPIPSAFCFLSHDHGRTWARGHFVAQDTLECQVAEVETGEQRVVTLNARSHLRFRVQAQSTNDGLDFQESQLVKKLVEPPPTGCQGSVISFPSPRSGPGSPAQWLLYTHPTHSWQRADLGAYLNPRPPAPEAWSEPVLLAKGSAAYSDLQSMGTGPDGSPLFGCLYEANDYEEIVFLMFTLKQAFPAEYLPQ

SEQ ID NO: 29 - protein, 531 aa, synthetic construct
DASLPYLQKESVFQSGAHAYRIPALLYLPGQQSLLAFAEQRRSKKDEHAELIVLRRGDYDAGTHQVQWQAQEVVAQARLDGHRSMNPCPLYDEQTGTLFLFFIAIPGQVTEQQQLQTRANVTRLCYVTSTDHGRTWSSPRDLTDAAIGPAYREWSTFAVGPGHCLQLHDRARSLVVPAYAYRKLHPKQRPIPSAFCFLSHDHGRTWARGHFVAQDTLECQVAEVETGEQRVVTLNARSHLRFRVQAQSTNDGLDFQESQLVKKLVEPPPTGCQGSVISFPSPRSGPGSPAQWLLYTHPTHSWQRADLGAYLNPRPPAPEAWSEPVLLAKGSAAYSDLQSMGTGPDGSPLFGCLYEANDYEEIVFLMFTLKQAFPAEYLPQGGGGSGGGGSGGGGSGGGGSGGGGSQVQLVESGGGLVQAGGSLNLSCAVSDIMFSWSTMGWYRQAPGKERELVAQERGSGRINYADFVKGRFTISRDSAKNTMNLQMNSLKPEDTGVYYCWVRRPSGSWRGQHYPDAQEYWGQGTQVTVSS

SEQ ID NO: 30 - protein, 531 aa, synthetic construct
QVQLVESGGGLVQAGGSLNLSCAVSDIMFSWSTMGWYRQAPGKERELVAQERGSGRINYADFVKGRFTISRDSAKNTMNLQMNSLKPEDTGVYYCWVRRPSGSWRGQHYPDAQEYWGQGTQVTVSSGGGGSGGGGSGGGGSGGGGSGGGGSDASLPYLQKESVFQSGAHAYRIPALLYLPGQQSLLAFAEQRRSKKDEHAELIVLRRGDYDAGTHQVQWQAQEVVAQARLDGHRSMNPCPLYDEQTGTLFLFFIAIPGQVTEQQQLQTRANVTRLCYVTSTDHGRTWSSPRDLTDAAIGPAYREWSTFAVGPGHCLQLHDRARSLVVPAYAYRKLHPKQRPIPSAFCFLSHDHGRTWARGHFVAQDTLECQVAEVETGEQRVVTLNARSHLRFRVQAQSTNDGLDFQESQLVKKLVEPPPTGCQGSVISFPSPRSGPGSPAQWLLYTHPTHSWQRADLGAYLNPRPPAPEAWSEPVLLAKGSAAYSDLQSMGTGPDGSPLFGCLYEANDYEEIVFLMFTLKQAFPAEYLPQ

SEQ ID NO: 31 - protein, 5 aa, synthetic construct
WSTMG

SEQ ID NO: 32 - protein, 16 aa, synthetic construct
QERGSGRINYADFVKG

SEQ ID NO: 33 - protein, 18 aa, synthetic construct
RRPSGSWRGQHYPDAQEY

SEQ ID NO: 34 - protein, 33 aa, synthetic construct
FNMLQQRRFYEALHDPNLNEEQRNAKIKKIRDD

SEQ ID NO: 35 - protein, 33 aa, synthetic construct
LNMLQQRRFYEALHDPNLNEEQRNAKIKSIRDD

SEQ ID NO: 36 - protein, 33 aa, synthetic construct
FNMLQQRRFYEALHDPNLNEEQRNAKIKQIRDD

SEQ ID NO: 37 - protein, 33 aa, synthetic construct
LNMQQQRRFYEALHDPNLNEEQRNAKIKQIRDD

SEQ ID NO: 38 - protein, 33 aa, synthetic construct
FNMLQQRRFYEALHDPNLNEEQRNAKIKSIRDD

SEQ ID NO: 39 - protein, 33 aa, synthetic construct
FNMQQQRRFYEALHDPNLNEEQRNAKIKQIRDD

SEQ ID NO: 40 - protein, 33 aa, synthetic construct
FNMQQWRRFYEALHDPNLNEEQRNAKIKKIRDD

SEQ ID NO: 41 - protein, 33 aa, synthetic construct
LNMQQWRRFYEALHDPNLNEEQRNAKIKSIRDD

SEQ ID NO: 42 - protein, 249 aa, synthetic construct
EVQLLESGGGLVQPGGSLRLSCAASGFTFSSYAMSWVRQAPGKGLEWVSAISGSGGSTYYADSVKGRFTISRDNSKNTLYLQMNSLRAEDTAVYYCAKDFSSRRWYLEYWGQGTLVTVSSGGGGSGGGGSGGGGSGGGGSSSELTQDPAVSVALGQTVRITCQGDSLRSYYASWYQQKPGQAPVLVIYGKNNRPSGIPDRFSGSSSGNTASLTITGAQAEDEADYYCNSLERIGYLSYVFGGGTKLTVL

SEQ ID NO: 43 - protein, 307 aa, synthetic construct
EVQLLESGGGLVQPGGSLRLSCAASGFTFSSYAMSWVRQAPGKGLEWVSAISGSGGSTYYADSVKGRFTISRDNSKNTLYLQMNSLRAEDTAVYYCAKDFSSRRWYLEYWGQGTLVTVSSGGGGSGGGGSGGGGSGGGGSSSELTQDPAVSVALGQTVRITCQGDSLRSYYASWYQQKPGQAPVLVIYGKNNRPSGIPDRFSGSSSGNTASLTITGAQAEDEADYYCNSLERIGYLSYVFGGGTKLTVLGGGGSGGGGSGGGGSGGGGSGGGGSFNMLQQRRFYEALHDPNLNEEQRNAKIKSIRDD

SEQ ID NO: 44 - protein, 307 aa, synthetic construct
EVQLLESGGGLVQPGGSLRLSCAASGFTFSSYAMSWVRQAPGKGLEWVSAISGSGGSTYYADSVKGRFTISRDNSKNTLYLQMNSLRAEDTAVYYCAKDFSSRRWYLEYWGQGTLVTVSSGGGGSGGGGSGGGGSGGGGSSSELTQDPAVSVALGQTVRITCQGDSLRSYYASWYQQKPGQAPVLVIYGKNNRPSGIPDRFSGSSSGNTASLTITGAQAEDEADYYCNSLERIGYLSYVFGGGTKLTVLGGGGSGGGGSGGGGSGGGGSGGGGSLNMQQQRRFYEALHDPNLNEEQRNAKIKSIRDD

SEQ ID NO: 45 - protein, 307 aa, synthetic construct
EVQLLESGGGLVQPGGSLRLSCAASGFTFSSYAMSWVRQAPGKGLEWVSAISGSGGSTYYADSVKGRFTISRDNSKNTLYLQMNSLRAEDTAVYYCAKDFSSRRWYLEYWGQGTLVTVSSGGGGSGGGGSGGGGSGGGGSSSELTQDPAVSVALGQTVRITCQGDSLRSYYASWYQQKPGQAPVLVIYGKNNRPSGIPDRFSGSSSGNTASLTITGAQAEDEADYYCNSLERIGYLSYVFGGGTKLTVLGGGGSGGGGSGGGGSGGGGSGGGGSFNMQQQRRFYEALHDPNLNEEQRNAKIKQIRDD

SEQ ID NO: 46 - protein, 307 aa, synthetic construct
EVQLLESGGGLVQPGGSLRLSCAASGFTFSSYAMSWVRQAPGKGLEWVSAISGSGGSTYYADSVKGRFTISRDNSKNTLYLQMNSLRAEDTAVYYCAKDFSSRRWYLEYWGQGTLVTVSSGGGGSGGGGSGGGGSGGGGSSSELTQDPAVSVALGQTVRITCQGDSLRSYYASWYQQKPGQAPVLVIYGKNNRPSGIPDRFSGSSSGNTASLTITGAQAEDEADYYCNSLERIGYLSYVFGGGTKLTVLGGGGSGGGGSGGGGSGGGGSGGGGSFNMQQWRRFYEALHDPNLNEEQRNAKIKSIRDD

SEQ ID NO: 47 - protein, 307 aa, synthetic construct
EVQLLESGGGLVQPGGSLRLSCAASGFTFSSYAMSWVRQAPGKGLEWVSAISGSGGSTYYADSVKGRFTISRDNSKNTLYLQMNSLRAEDTAVYYCAKDFSSRRWYLEYWGQGTLVTVSSGGGGSGGGGSGGGGSGGGGSSSELTQDPAVSVALGQTVRITCQGDSLRSYYASWYQQKPGQAPVLVIYGKNNRPSGIPDRFSGSSSGNTASLTITGAQAEDEADYYCNSLERIGYLSYVFGGGTKLTVLGGGGSGGGGSGGGGSGGGGSGGGGSFNMQQQRRFYEALHDPNLNEEQRNAKIKSIRDD

SEQ ID NO: 48 - protein, 307 aa, synthetic construct
EVQLLESGGGLVQPGGSLRLSCAASGFTFSSYAMSWVRQAPGKGLEWVSAISGSGGSTYYADSVKGRFTISRDNSKNTLYLQMNSLRAEDTAVYYCAKDFSSRRWYLEYWGQGTLVTVSSGGGGSGGGGSGGGGSGGGGSSSELTQDPAVSVALGQTVRITCQGDSLRSYYASWYQQKPGQAPVLVIYGKNNRPSGIPDRFSGSSSGNTASLTITGAQAEDEADYYCNSLERIGYLSYVFGGGTKLTVLGGGGSGGGGSGGGGSGGGGSGGGGSFNMQQQRRFYEALHDALMNEEQRNAKIKSIRDD

SEQ ID NO: 49 - protein, 307 aa, synthetic construct
EVQLLESGGGLVQPGGSLRLSCAASGFTFSSYAMSWVRQAPGKGLEWVSAISGSGGSTYYADSVKGRFTISRDNSKNTLYLQMNSLRAEDTAVYYCAKDFSSRRWYLEYWGQGTLVTVSSGGGGSGGGGSGGGGSGGGGSSSELTQDPAVSVALGQTVRITCQGDSLRSYYASWYQQKPGQAPVLVIYGKNNRPSGIPDRFSGSSSGNTASLTITGAQAEDEADYYCNSLERIGYLSYVFGGGTKLTVLGGGGSGGGGSGGGGSGGGGSGGGGSFNMQQQRRFYEALHDALMNEEQRNAKIKRIRDD

SEQ ID NO: 50 - protein, 307 aa, synthetic construct
EVQLLESGGGLVQPGGSLRLSCAASGFTFSSYAMSWVRQAPGKGLEWVSAISGSGGSTYYADSVKGRFTISRDNSKNTLYLQMNSLRAEDTAVYYCAKDFSSRRWYLEYWGQGTLVTVSSGGGGSGGGGSGGGGSGGGGSSSELTQDPAVSVALGQTVRITCQGDSLRSYYASWYQQKPGQAPVLVIYGKNNRPSGIPDRFSGSSSGNTASLTITGAQAEDEADYYCNSLERIGYLSYVFGGGTKLTVLGGGGSGGGGSGGGGSGGGGSGGGGSFNMQQQRRFYEALHDALMNEEQRNAKIKNIRDD

SEQ ID NO: 51 - protein, 307 aa, synthetic construct
EVQLLESGGGLVQPGGSLRLSCAASGFTFSSYAMSWVRQAPGKGLEWVSAISGSGGSTYYADSVKGRFTISRDNSKNTLYLQMNSLRAEDTAVYYCAKDFSSRRWYLEYWGQGTLVTVSSGGGGSGGGGSGGGGSGGGGSSSELTQDPAVSVALGQTVRITCQGDSLRSYYASWYQQKPGQAPVLVIYGKNNRPSGIPDRFSGSSSGNTASLTITGAQAEDEADYYCNSLERIGYLSYVFGGGTKLTVLGGGGSGGGGSGGGGSGGGGSGGGGSFNMQQQRRFYETLWDLTLNEEQRNAKIKSIRDD

SEQ ID NO: 52 - protein, 307 aa, synthetic construct
EVQLLESGGGLVQPGGSLRLSCAASGFTFSSYAMSWVRQAPGKGLEWVSAISGSGGSTYYADSVKGRFTISRDNSKNTLYLQMNSLRAEDTAVYYCAKDFSSRRWYLEYWGQGTLVTVSSGGGGSGGGGSGGGGSGGGGSSSELTQDPAVSVALGQTVRITCQGDSLRSYYASWYQQKPGQAPVLVIYGKNNRPSGIPDRFSGSSSGNTASLTITGAQAEDEADYYCNSLERIGYLSYVFGGGTKLTVLGGGGSGGGGSGGGGSGGGGSGGGGSFNMQQQRRFYETLWDLTLNEEQRNAKIKKIRDD

SEQ ID NO: 53 - protein, 307 aa, synthetic construct
EVQLLESGGGLVQPGGSLRLSCAASGFTFSSYAMSWVRQAPGKGLEWVSAISGSGGSTYYADSVKGRFTISRDNSKNTLYLQMNSLRAEDTAVYYCAKDFSSRRWYLEYWGQGTLVTVSSGGGGSGGGGSGGGGSGGGGSSSELTQDPAVSVALGQTVRITCQGDSLRSYYASWYQQKPGQAPVLVIYGKNNRPSGIPDRFSGSSSGNTASLTITGAQAEDEADYYCNSLERIGYLSYVFGGGTKLTVLGGGGSGGGGSGGGGSGGGGSGGGGSFNMQQQRRFYDALHDLLLNEEQRNAKIKSIRDD

SEQ ID NO: 54 - protein, 307 aa, synthetic construct
EVQLLESGGGLVQPGGSLRLSCAASGFTFSSYAMSWVRQAPGKGLEWVSAISGSGGSTYYADSVKGRFTISRDNSKNTLYLQMNSLRAEDTAVYYCAKDFSSRRWYLEYWGQGTLVTVSSGGGGSGGGGSGGGGSGGGGSSSELTQDPAVSVALGQTVRITCQGDSLRSYYASWYQQKPGQAPVLVIYGKNNRPSGIPDRFSGSSSGNTASLTITGAQAEDEADYYCNSLERIGYLSYVFGGGTKLTVLGGGGSGGGGSGGGGSGGGGSGGGGSFNMLQQRRFYDALHDLLLNEEQRNAKIKSIRDD

SEQ ID NO: 55 - protein, 364 aa, synthetic construct
ENDFGLVQPLVTMEQLLWVSGRQIGSVDTFRIPLITATPRGTLLAFAEARKMSSSDEGAKFIALRRSMDQGSTWSPTAFIVNDGDVPDGLNLGAVVSDVETGVVFLFYSLCAHKAGCQVASTMLVWSKDDGVSWSTPRNLSLDIGTEVFAPGPGSGIQKQREPRKGRLIVCGHGTLERDGVFCLLSDDHGASWRYGSGVSGIPYGQPKQENDFNPDECQPYELPDGSVVINARNQNNYHCHCRIVLRSYDACDTLRPRDVTFDPELVDPVVAAGAVVTSSGIVFFSNPAHPEFRVNLTLRWSFSNGTSWRKETVQLWPGPSGYSSLATLEGSMDGEEQAPQLYVLYEKGRNHYTESISVAKISV

SEQ ID NO: 56 - protein, 380 aa, synthetic construct
MASLPVLQKESVFQSGAHAYRIPALLYLPGQQSLLAFAEQRASKKDEHAELIVLRRGDYDAPTHQVQWQAQEVVAQARLDGHRSMNPCPLYDAQTGTLFLFFIAIPGQVTEQQQLQTRANVTRLCQVTSTDHGRTWSSPRDLTDAAIGPAYREWSTFAVGPGHCLQLHDRARSLVVPAYAYRKLHPIQRPIPSAFCFLSHDHGRTWARGHFVAQDTLECQVAEVETGEQRVVTLNARSHLRARVQAQSTNDGLDFQESQLVKKLVEPPPQGCQGSVISFPSPRSGPGSPAQWLLYTHPTHSWQRADLGAYLNPRPPAPEAWSEPVLLAKGSCAYSDLQSMGTGPDGSPLFGCLYEANDYEEIVFLMFTLKQAFPAEYLPQ

SEQ ID NO: 57 - protein, 428 aa, synthetic construct
MEEVTTCSFNSPLFRQEDDRGITYRIPALLYIPPTHTFLAFAEKRSTRRDEDALHLVLRRGLRIGQLVQWGPLKPLMEATLPGHRTMNPCPVWEQKSGCVFLFFICVRGHVTERQQIVSGRNAARLCFIYSQDAGCSWSEVRDLTEEVIGSELKHWATFAVGPGHGIQLQSGRLVIPAYTYYIPSWFFCFQLPCKTRPHSLMIYSDDLGVTWHHGRLIRPMVTVECEVAEVTGRAGHPVLYCSARTPNRCRAEALSTDHGEGFQRLALSRQLCEPPHGCQGSVVSFRPLEIPHRCQDSSSKDAPTIQQSSPGSSLRLEEEAGTPSESWLLYSHPTSRKQRVDLGIYLNQTPLEAACWSRPWILHCGPCGYSDLAALEEEGLFGCLFECGTKQECEQIAFRLFTHREILSHLQGDCTSPGRNPSQFKSN

SEQ ID NO: 58 - protein, 461 aa, synthetic construct
MRPADLPPRPMEESPASSSAPTETEEPGSSAEVMEEVTTCSFNSPLFRQEDDRGITYRIPALLYIPPTHTFLAFAEKRSTRRDEDALHLVLRRGLRIGQLVQWGPLKPLMEATLPGHRTMNPCPVWEQKSGCVFLFFICVRGHVTERQQIVSGRNAARLCFIYSQDAGCSWSEVRDLTEEVIGSELKHWATFAVGPGHGIQLQSGRLVIPAYTYYIPSWFFCFQLPCKTRPHSLMIYSDDLGVTWHHGRLIRPMVTVECEVAEVTGRAGHPVLYCSARTPNRCRAEALSTDHGEGFQRLALSRQLCEPPHGCQGSVVSFRPLEIPHRCQDSSSKDAPTIQQSSPGSSLRLEEEAGTPSESWLLYSHPTSRKQRVDLGIYLNQTPLEAACWSRPWILHCGPCGYSDLAALEEEGLFGCLFECGTKQECEQIAFRLFTHREILSHLQGDCTSPGRNPSQFKSN

SEQ ID NO: 59 - protein, 484 aa, synthetic construct
MGVPRTPSRTVLFERERTGLTYRVPSLLPVPPGPTLLAFVEQRLSPDDSHAHRLVLRRGTLAGGSVRWGALHVLGTAALAEHRSMNPCPVHDAGTGTVFLFFIAVLGHTPEAVQIATGRNAARLCCVASRDAGLSWGSARDLTEEAIGGAVQDWATFAVGPGHGVQLPSGRLLVPAYTYRVDRRECFGKICRTSPHSFAFYSDDHGRTWRCGGLVPNLRSGECQLAAVDGGQAGSFLYCNARSPLGSRVQALSTDEGTSFLPAERVASLPETAWGCQGSIVGFPAPAPNRPRDDSWSVGPGSPLQPPLLGPGVHEPPEEAAVDPRGGQVPGGPFSRLQPRGDGPRQPGPRPGVSGDVGSWTLALPMPFAAPPQSPTWLLYSHPVGRRARLHMGIRLSQSPLDPRSWTEPWVIYEGPSGYSDLASIGPAPEGGLVFACLYESGARTSYDEISFCTFSLREVLENVPASPKPPNLGDKPRGCCWPS

SEQ ID NO: 60 - protein, 496 aa, synthetic construct
MMSSAAFPRWLSMGVPRTPSRTVLFERERTGLTYRVPSLLPVPPGPTLLAFVEQRLSPDDSHAHRLVLRRGTLAGGSVRWGALHVLGTAALAEHRSMNPCPVHDAGTGTVFLFFIAVLGHTPEAVQIATGRNAARLCCVASRDAGLSWGSARDLTEEAIGGAVQDWATFAVGPGHGVQLPSGRLLVPAYTYRVDRRECFGKICRTSPHSFAFYSDDHGRTWRCGGLVPNLRSGECQLAAVDGGQAGSFLYCNARSPLGSRVQALSTDEGTSFLPAERVASLPETAWGCQGSIVGFPAPAPNRPRDDSWSVGPGSPLQPPLLGPGVHEPPEEAAVDPRGGQVPGGPFSRLQPRGDGPRQPGPRPGVSGDVGSWTLALPMPFAAPPQSPTWLLYSHPVGRRARLHMGIRLSQSPLDPRSWTEPWVIYEGPSGYSDLASIGPAPEGGLVFACLYESGARTSYDEISFCTFSLREVLENVPASPKPPNLGDKPRGCCWPS

SEQ ID NO: 61 - protein, 505 aa, synthetic construct
FNMQQQRRFYEALHDPNLNEEQRNAKIKQIRDDGGGGSGGGGSGGGGSGGGGSGGGGSLNFRAPPVIPNVPFLWAWNAPSEFCLGKFDEPLDMSLFSFIGSPRINATGQGVTIFYVDRLGYYPYIDSITGVTVNGGIPQKISLQDHLDKAKKDITFYMPVDNLGMAVIDWEEWRPTWARNWKPKDVYKNRSIELVQQQNVQLSLTEATEKAKQEFEKAGKDFLVETIKLGKLLRPNHLWGYYLFPDCYNHHYKKPGYNGSCFNVEIKRNDDLSWLWNESTALYPSIYLNTQQSPVAATLYVRNRVREAIRVSKIPDAKSPLPVFAYTRIVFTDQVLKFLSQDELVYTFGETVALGASGIVIWGTLSIMRSMKSCLLLDNYMETILNPYIINVTLAAKMCSQVLCQEQGVCIRKNWNSSDYLHLNPDNFAIQLEKGGKFTVRGKPTLEDLEQFSEKFYCSCYSTLSCKEKADVKDTDAVDVCIADGVCIDAFLKPPMETEEPQIFY

SEQ ID NO: 62 - protein, 505 aa, synthetic construct
LNFRAPPVIPNVPFLWAWNAPSEFCLGKFDEPLDMSLFSFIGSPRINATGQGVTIFYVDRLGYYPYIDSITGVTVNGGIPQKISLQDHLDKAKKDITFYMPVDNLGMAVIDWEEWRPTWARNWKPKDVYKNRSIELVQQQNVQLSLTEATEKAKQEFEKAGKDFLVETIKLGKLLRPNHLWGYYLFPDCYNHHYKKPGYNGSCFNVEIKRNDDLSWLWNESTALYPSIYLNTQQSPVAATLYVRNRVREAIRVSKIPDAKSPLPVFAYTRIVFTDQVLKFLSQDELVYTFGETVALGASGIVIWGTLSIMRSMKSCLLLDNYMETILNPYIINVTLAAKMCSQVLCQEQGVCIRKNWNSSDYLHLNPDNFAIQLEKGGKFTVRGKPTLEDLEQFSEKFYCSCYSTLSCKEKADVKDTDAVDVCIADGVCIDAFLKPPMETEEPQIFYGGGGSGGGGSGGGGSGGGGSGGGGSFNMQQQRRFYEALHDPNLNEEQRNAKIKQIRDD

SEQ ID NO: 63 - protein, 505 aa, synthetic construct
FNMLQQRRFYEALHDPNLNEEQRNAKIKSIRDDGGGGSGGGGSGGGGSGGGGSGGGGSLNFRAPPVIPNVPFLWAWNAPSEFCLGKFDEPLDMSLFSFIGSPRINATGQGVTIFYVDRLGYYPYIDSITGVTVNGGIPQKISLQDHLDKAKKDITFYMPVDNLGMAVIDWEEWRPTWARNWKPKDVYKNRSIELVQQQNVQLSLTEATEKAKQEFEKAGKDFLVETIKLGKLLRPNHLWGYYLFPDCYNHHYKKPGYNGSCFNVEIKRNDDLSWLWNESTALYPSIYLNTQQSPVAATLYVRNRVREAIRVSKIPDAKSPLPVFAYTRIVFTDQVLKFLSQDELVYTFGETVALGASGIVIWGTLSIMRSMKSCLLLDNYMETILNPYIINVTLAAKMCSQVLCQEQGVCIRKNWNSSDYLHLNPDNFAIQLEKGGKFTVRGKPTLEDLEQFSEKFYCSCYSTLSCKEKADVKDTDAVDVCIADGVCIDAFLKPPMETEEPQIFY

SEQ ID NO: 64 - protein, 505 aa, synthetic construct
LNFRAPPVIPNVPFLWAWNAPSEFCLGKFDEPLDMSLFSFIGSPRINATGQGVTIFYVDRLGYYPYIDSITGVTVNGGIPQKISLQDHLDKAKKDITFYMPVDNLGMAVIDWEEWRPTWARNWKPKDVYKNRSIELVQQQNVQLSLTEATEKAKQEFEKAGKDFLVETIKLGKLLRPNHLWGYYLFPDCYNHHYKKPGYNGSCFNVEIKRNDDLSWLWNESTALYPSIYLNTQQSPVAATLYVRNRVREAIRVSKIPDAKSPLPVFAYTRIVFTDQVLKFLSQDELVYTFGETVALGASGIVIWGTLSIMRSMKSCLLLDNYMETILNPYIINVTLAAKMCSQVLCQEQGVCIRKNWNSSDYLHLNPDNFAIQLEKGGKFTVRGKPTLEDLEQFSEKFYCSCYSTLSCKEKADVKDTDAVDVCIADGVCIDAFLKPPMETEEPQIFYGGGGSGGGGSGGGGSGGGGSGGGGSFNMLQQRRFYEALHDPNLNEEQRNAKIKSIRDD

SEQ ID NO: 65 - protein, 446 aa, synthetic construct
LNFRAPPVIPNVPFLWAWNAPSEFCLGKFDEPLDMSLFSFIGSPRINATGQGVTIFYVDRLGYYPYIDSITGVTVNGGIPQKISLQDHLDKAKKDITFYMPVDNLGMAVIDWEEWRPTWARNWKPKDVYKNRSIELVQQQNVQLSLTEATEKAKQEFEKAGKDFLVETIKLGKLLRPNHLWGYYLFPDCYNHHYKKPGYNGSCFNVEIKRNDDLSWLWNESTALYPSIYLNTQQSPVAATLYVRNRVREAIRVSKIPDAKSPLPVFAYTRIVFTDQVLKFLSQDELVYTFGETVALGASGIVIWGTLSIMRSMKSCLLLDNYMETILNPYIINVTLAAKMCSQVLCQEQGVCIRKNWNSSDYLHLNPDNFAIQLEKGGKFTVRGKPTLEDLEQFSEKFYCSCYSTLSCKEKADVKDTDAVDVCIADGVCIDAFLKPPMETEEPQIF

SEQ ID NO: 66 - protein, 445 aa, synthetic construct
LNFRAPPVIPNVPFLWAWNAPSEFCLGKFDEPLDMSLFSFIGSPRINATGQGVTIFYVDRLGYYPYIDSITGVTVNGGIPQKISLQDHLDKAKKDITFYMPVDNLGMAVIDWEEWRPTWARNWKPKDVYKNRSIELVQQQNVQLSLTEATEKAKQEFEKAGKDFLVETIKLGKLLRPNHLWGYYLFPDCYNHHYKKPGYNGSCFNVEIKRNDDLSWLWNESTALYPSIYLNTQQSPVAATLYVRNRVREAIRVSKIPDAKSPLPVFAYTRIVFTDQVLKFLSQDELVYTFGETVALGASGIVIWGTLSIMRSMKSCLLLDNYMETILNPYIINVTLAAKMCSQVLCQEQGVCIRKNWNSSDYLHLNPDNFAIQLEKGGKFTVRGKPTLEDLEQFSEKFYCSCYSTLSCKEKADVKDTDAVDVCIADGVCIDAFLKPPMETEEPQI

SEQ ID NO: 67 - protein, 444 aa, synthetic construct
LNFRAPPVIPNVPFLWAWNAPSEFCLGKFDEPLDMSLFSFIGSPRINATGQGVTIFYVDRLGYYPYIDSITGVTVNGGIPQKISLQDHLDKAKKDITFYMPVDNLGMAVIDWEEWRPTWARNWKPKDVYKNRSIELVQQQNVQLSLTEATEKAKQEFEKAGKDFLVETIKLGKLLRPNHLWGYYLFPDCYNHHYKKPGYNGSCFNVEIKRNDDLSWLWNESTALYPSIYLNTQQSPVAATLYVRNRVREAIRVSKIPDAKSPLPVFAYTRIVFTDQVLKFLSQDELVYTFGETVALGASGIVIWGTLSIMRSMKSCLLLDNYMETILNPYIINVTLAAKMCSQVLCQEQGVCIRKNWNSSDYLHLNPDNFAIQLEKGGKFTVRGKPTLEDLEQFSEKFYCSCYSTLSCKEKADVKDTDAVDVCIADGVCIDAFLKPPMETEEPQ

SEQ ID NO: 68 - protein, 443 aa, synthetic construct
LNFRAPPVIPNVPFLWAWNAPSEFCLGKFDEPLDMSLFSFIGSPRINATGQGVTIFYVDRLGYYPYIDSITGVTVNGGIPQKISLQDHLDKAKKDITFYMPVDNLGMAVIDWEEWRPTWARNWKPKDVYKNRSIELVQQQNVQLSLTEATEKAKQEFEKAGKDFLVETIKLGKLLRPNHLWGYYLFPDCYNHHYKKPGYNGSCFNVEIKRNDDLSWLWNESTALYPSIYLNTQQSPVAATLYVRNRVREAIRVSKIPDAKSPLPVFAYTRIVFTDQVLKFLSQDELVYTFGETVALGASGIVIWGTLSIMRSMKSCLLLDNYMETILNPYIINVTLAAKMCSQVLCQEQGVCIRKNWNSSDYLHLNPDNFAIQLEKGGKFTVRGKPTLEDLEQFSEKFYCSCYSTLSCKEKADVKDTDAVDVCIADGVCIDAFLKPPMETEEP

SEQ ID NO: 69 - protein, 439 aa, synthetic construct
LNFRAPPVIPNVPFLWAWNAPSEFCLGKFDEPLDMSLFSFIGSPRINATGQGVTIFYVDRLGYYPYIDSITGVTVNGGIPQKISLQDHLDKAKKDITFYMPVDNLGMAVIDWEEWRPTWARNWKPKDVYKNRSIELVQQQNVQLSLTEATEKAKQEFEKAGKDFLVETIKLGKLLRPNHLWGYYLFPDCYNHHYKKPGYNGSCFNVEIKRNDDLSWLWNESTALYPSIYLNTQQSPVAATLYVRNRVREAIRVSKIPDAKSPLPVFAYTRIVFTDQVLKFLSQDELVYTFGETVALGASGIVIWGTLSIMRSMKSCLLLDNYMETILNPYIINVTLAAKMCSQVLCQEQGVCIRKNWNSSDYLHLNPDNFAIQLEKGGKFTVRGKPTLEDLEQFSEKFYCSCYSTLSCKEKADVKDTDAVDVCIADGVCIDAFLKPPME

SEQ ID NO: 70 - protein, 438 aa, synthetic construct
LNFRAPPVIPNVPFLWAWNAPSEFCLGKFDEPLDMSLFSFIGSPRINATGQGVTIFYVDRLGYYPYIDSITGVTVNGGIPQKISLQDHLDKAKKDITFYMPVDNLGMAVIDWEEWRPTWARNWKPKDVYKNRSIELVQQQNVQLSLTEATEKAKQEFEKAGKDFLVETIKLGKLLRPNHLWGYYLFPDCYNHHYKKPGYNGSCFNVEIKRNDDLSWLWNESTALYPSIYLNTQQSPVAATLYVRNRVREAIRVSKIPDAKSPLPVFAYTRIVFTDQVLKFLSQDELVYTFGETVALGASGIVIWGTLSIMRSMKSCLLLDNYMETILNPYIINVTLAAKMCSQVLCQEQGVCIRKNWNSSDYLHLNPDNFAIQLEKGGKFTVRGKPTLEDLEQFSEKFYCSCYSTLSCKEKADVKDTDAVDVCIADGVCIDAFLKPPM

SEQ ID NO: 71 - protein, 431 aa, synthetic construct
FRAPPVIPNVPFLWAWNAPSEFCLGKFDEPLDMSLFSFIGSPRINATGQGVTIFYVDRLGYYPYIDSITGVTVNGGIPQKISLQDHLDKAKKDITFYMPVDNLGMAVIDWEEWRPTWARNWKPKDVYKNRSIELVQQQNVQLSLTEATEKAKQEFEKAGKDFLVETIKLGKLLRPNHLWGYYLFPDCYNHHYKKPGYNGSCFNVEIKRNDDLSWLWNESTALYPSIYLNTQQSPVAATLYVRNRVREAIRVSKIPDAKSPLPVFAYTRIVFTDQVLKFLSQDELVYTFGETVALGASGIVIWGSWENTRTKESCQAIKEYMDTTLNPYIINVTLAAKMCSQVLCQEQGVCIRKNWNSSDYLHLNPDNFAIQLEKGGKFTVRGKPTLEDLEQFSEKFYCSCYSTLSCKEKADVKDTDAVDVCIADGVCIDAF